European Patent Application EP 4 455 264 A1, published October 30, 2024. Title: Method for Producing Carbohydrates Containing Lacto-N-Triose II as Core Trisaccharide and Method for Producing Crystals of the Carbohydrates. Applicant: 協和発酵バイオ株式会社. The sequence listing filed with the application follows.

SEQUENCE LISTING (67 sequences)

SEQ ID NO: 1 - DNA, 1191 bp, Escherichia coli
  source 1..1191: mol_type = genomic DNA
atgacaacaaacactgtttcccgcaaagtggcgtggctacgggtcgttacgctggcagtcgccgccttcatcttcaacaccaccgaatttgtccctgttggcctgctctctgacattgcgcaaagttttcacatgcaaaccgctcaggtcggcatcatgttgaccatttacgcatgggtagtagcgctaatgtcattgccttttatgttaatgaccagtcaggttgaacggcgcaaattactgatctgcctgtttgtggtgtttattgccagccacgtactgtcgtttttgtcgtggagctttaccgttctggtgatcagtcgcattggtgtggcttttgcacatgcgattttctggtcgattacggcgtctctggcgatccgtatggctccggccgggaagcgagcacaggcattgagtttaattgccaccggtacagcactggcgatggtcttaggtttacctctcgggcgcattgtgggccagtatttcggttggcgaatgaccttcttcgcgattggtattggggcgcttatcacccttttgtgcctgattaagttacttcccttactgcccagtgagcattccggttcactgaaaagcctcccgctattgttccgccgcccggcattgatgagcatttatttgttaactgtggtggttgtcaccgcccattacacggcatacagctatatcgagccttttgtacaaaacattgcgggattcagcgccaactttgccacggcattactgttattactcggtggtgcgggcattattggcagcgtgattttcggtaaactgggtaatcagtatgcgtctgcgttggtgagtacggcgattgcgctgttgctggtgtgcctggcattgctgttacctgcggcgaacagtgaaatacacctcggggtgctgagtattttctgggggatcgcgatgatgatcatcgggcttggtatgcaggttaaagtgctggcgctggcaccagatgctaccgacgtcgcgatggcgctattctccggcatatttaatattggaatcggggcgggtgcgttggtaggtaatcaggtgagtttgcactggtcaatgtcgatgattggttatgtgggcgcggtgcctgcttttgccgcgttaatttggtcaatcattatatttcgccgctggccagtgacactcgaagaacagacgcaatag

SEQ ID NO: 2 - protein, 396 aa, Escherichia coli
MTTNTVSRKVAWLRVVTLAVAAFIFNTTEFVPVGLLSDIAQSFHMQTAQVGIMLTIYAWVVALMSLPFMLMTSQVERRKLLICLFVVFIASHVLSFLSWSFTVLVISRIGVAFAHAIFWSITASLAIRMAPAGKRAQALSLIATGTALAMVLGLPLGRIVGQYFGWRMTFFAIGIGALITLLCLIKLLPLLPSEHSGSLKSLPLLFRRPALMSIYLLTVVVVTAHYTAYSYIEPFVQNIAGFSANFATALLLLLGGAGIIGSVIFGKLGNQYASALVSTAIALLLVCLALLLPAANSEIHLGVLSIFWGIAMMIIGLGMQVKVLALAPDATDVAMALFSGIFNIGIGAGALVGNQVSLHWSMSMIGYVGAVPAFAALIWSIIIFRRWPVTLEEQTQ

SEQ ID NO: 3 - DNA, 1233 bp, Escherichia coli
  source 1..1233: mol_type = genomic DNA
atgcaaaataaattagcttccggtgccaggcttggacgtcaggcgttacttttccctctctgtctggtgctttacgaattttcaacctatatcggcaacgatatgattcaacccggtatgttggccgtggtggaacaatatcaggcgggcattgattgggttcctacttcgatgaccgcgtatctggcgggcgggatgtttttacaatggctgctggggccgctgtcggatcgtattggtcgccgtccggtgatgctggcgggagtggtgtggtttatcgtcacctgtctggcaatattgctggcgcaaaacattgaacaattcaccctgttgcgcttcttgcagggcataagcctctgtttcattggcgctgtgggatacgccgcaattcaggaatccttcgaagaggcggtttgtatcaagatcaccgcgctgatggcgaacgtggcgctgattgctccgctacttggtccgctggtgggcgcggcgtggatccatgtgctgccctgggaggggatgtttgttttgtttgccgcattggcagcgatctcctttttcggtctgcaacgagccatgcctgaaaccgccacgcgtataggcgagaaactgtcactgaaagaactcggtcgtgactataagctggtgctgaagaacggccgctttgtggcgggggcgctggcgctgggattcgttagtctgccgttgctggcgtggatcgcccagtcgccgattatcatcattaccggcgagcagttgagcagctatgaatatggcttgctgcaagtgcctattttcggggcgttaattgcgggtaacttgctgttagcgcgtctgacctcgcgccgcaccgtacgttcgctgattattatgggcggctggccgattatgattggtctattggtcgctgctgcggcaacggttatctcatcgcacgcgtatttatggatgactgccgggttaagtatttatgctttcggtattggtctggcgaatgcgggactggtgcgattaaccctgtttgccagcgatatgagtaaaggtacggtttctgccgcgatgggaatgctgcaaatgctgatctttaccgttggtattgaaatcagcaaacatgcctggctgaacgggggcaacggactgtttaatctcttcaaccttgtcaacggaattttgtggctgtcgctgatggttatctttttaaaagataaacagatgggaaattctcacgaagggtaa

SEQ ID NO: 4 - protein, 410 aa, Escherichia coli
MQNKLASGARLGRQALLFPLCLVLYEFSTYIGNDMIQPGMLAVVEQYQAGIDWVPTSMTAYLAGGMFLQWLLGPLSDRIGRRPVMLAGVVWFIVTCLAILLAQNIEQFTLLRFLQGISLCFIGAVGYAAIQESFEEAVCIKITALMANVALIAPLLGPLVGAAWIHVLPWEGMFVLFAALAAISFFGLQRAMPETATRIGEKLSLKELGRDYKLVLKNGRFVAGALALGFVSLPLLAWIAQSPIIIITGEQLSSYEYGLLQVPIFGALIAGNLLLARLTSRRTVRSLIIMGGWPIMIGLLVAAAATVISSHAYLWMTAGLSIYAFGIGLANAGLVRLTLFASDMSKGTVSAAMGMLQMLIFTVGIEISKHAWLNGGNGLFNLFNLVNGILWLSLMVIFLKDKQMGNSHEG

SEQ ID NO: 5 - DNA, 1041 bp, Chromobacterium violaceum
  source 1..1041: mol_type = genomic DNA
atgcagccgctggtgagcgttctgatttgcgcgtacaacgtggagaagtattttgcgcaggcgctggatgcggtggttggtcaaacctggcgtaacctggacatcctgattgttgacgatggcagcaccgatggtaccctggcgatcgcgaaggactttcaaaaacgtgatagccgtatcaagattctggcgcaggcgcaaaacagcggcctgatcccgagcctgaacattggtctggatgagctggcgaaaagcggtggcggtgaatacattgcgcgtaccgatgcggatgatattgcggcgccggattggatcgagaagattgtgggcgagatggaaaaagaccgtagcatcattgcgatgggtgcgtggctggaagttctgagcgaggaaaaggatggcaaccgtctggcgcgtcaccacgagcacggtaaaatttggaagaaaccgacccgtcacgaagacatcgcggcgttctttccgttcggcaacccgatccacaacaacaccatgattatgcgtcgtagcgtgatcgacggcggtctgcgttacaacaccgagcgtgactgggcggaagattaccagttttggtatgatgttagcaagctgggtcgtctggcgtactatccggaggcgctggtgaagtatcgtctgcacgcgaaccaagttagcagcaaacacagcattcgtcaacacgaaatcgcgcagggcattcaaaagaccgcgcgtaacgacttcctgcagagcatgggtttcaaaacccgttttgatagcctggagtaccgtcaaaccaaggcggcggcgtatgagctgctggaaaaagacctgccggaggaagatttcgaacgtgcgcgtcgtttcctgtaccagtgctttaaacgtaccgacaccccgccggcgggtgcgtggctggactttgcggcggatggtcgtatgcgtcgtctgttcaccctgcgtcaatattttagcatcctgcaccgtctgattaagaaccgtcgtcaggcgcgtagcgatagcgcgggtaaagagcaagaaatctaa

SEQ ID NO: 6 - protein, 346 aa, Neisseria polysaccharea
MQPLVSVLICAYNVEKYFAQALDAVVGQTWRNLDILIVDDGSTDGTLAIAKDFQKRDSRIKILAQAQNSGLIPSLNIGLDELAKSGGGEYIARTDADDIAAPDWIEKIVGEMEKDRSIIAMGAWLEVLSEEKDGNRLARHHEHGKIWKKPTRHEDIAAFFPFGNPIHNNTMIMRRSVIDGGLRYNTERDWAEDYQFWYDVSKLGRLAYYPEALVKYRLHANQVSSKHSIRQHEIAQGIQKTARNDFLQSMGFKTRFDSLEYRQTKAAAYELLEKDLPEEDFERARRFLYQCFKRTDTPPAGAWLDFAADGRMRRLFTLRQYFSILHRLIKNRRQARSDSAGKEQEI

SEQ ID NO: 7 - DNA, 789 bp, Chromobacterium violaceum
  source 1..789: mol_type = genomic DNA
atggacaccatcatgattaaacgtccgctggttagcgttattctgccggtgaataaaaacaatccgcatctggaagaagcaatccagagcattaaaaaccagacctataaagagctggaactgatcattattgccaacaactgcgaggataacttttatagcctgctgctgaaatatcaggaccagaaaaccaaaattatccgcaccagcatcaaatatctgccgtttagcctgaatctgggtgttcatctgagccagggtgaatatattgcacgtatggattcagatgatatcagcgttctggatcgcattgaaaaacaggttaaacgctttctgaatacaccggaactgagcattctgggtagcaatgttgaatatatcaatgaagccagcgaaagcattggctatagcaactatccgctggatcatagcagcattgttaatagctttccgtttcgttgtaatctggcacatccgaccattatggttaaaaaagaagtgattaccacgcttggtggctatatgtatggtagcctgagcgaagattatgatctgtggattcgtgcaagccgtcatggcaatttcaaatttagcaatattgatgaaccgctgctgaagtaccgtattcataaaggtcaggcaaccaataaaagcaacgcctataacatctttgcctttgatagcagcctgaaaatccgtgaatttctgctgaatggtaatgtgcagtatctgctgggtgcagcacgtggtttttttgcatttctgtatgtgcgcttcatcaaaaaatga

SEQ ID NO: 8 - protein, 262 aa, Chromobacterium violaceum
MDTIMIKRPLVSVILPVNKNNPHLEEAIQSIKNQTYKELELIIIANNCEDNFYSLLLKYQDQKTKIIRTSIKYLPFSLNLGVHLSQGEYIARMDSDDISVLDRIEKQVKRFLNTPELSILGSNVEYINEASESIGYSNYPLDHSSIVNSFPFRCNLAHPTIMVKKEVITTLGGYMYGSLSEDYDLWIRASRHGNFKFSNIDEPLLKYRIHKGQATNKSNAYNIFAFDSSLKIREFLLNGNVQYLLGAARGFFAFLYVRFIKK

SEQ ID NO: 9 - DNA, 20 bp, synthetic construct
  misc_feature 1..20: note = Description of the artificial sequence: base sequence of primer for amplification of catsacB fragment
  source 1..20: mol_type = other DNA
accaggcgtttaagggcacc

SEQ ID NO: 10 - DNA, 21 bp, synthetic construct
  misc_feature 1..21: note = Description of the artificial sequence: base sequence of primer for amplification of catsacB fragment
  source 1..21: mol_type = other DNA
tacggttagccatttgcctgc

SEQ ID NO: 11 - DNA, 42 bp, synthetic construct
  misc_feature 1..42: note = Description of the artificial sequence: base sequence of primer for amplification of lacZ upstream 1
  source 1..42: mol_type = other DNA
ggtgcccttaaacgcctggtagctgtttcctgtgtgaaattg

SEQ ID NO: 12 - DNA, 18 bp, synthetic construct
  misc_feature 1..18: note = Description of the artificial sequence: base sequence of primer for amplification of lacZ upstream 1
  source 1..18: mol_type = other DNA
ccagtctggccctgcacg

SEQ ID NO: 13 - DNA, 43 bp, synthetic construct
  misc_feature 1..43: note = Description of the artificial sequence: base sequence of primer for amplification of lacY downstream 1
  source 1..43: mol_type = other DNA
gcaggcaaatggctaaccgtacgaccaacatatcataacggag

SEQ ID NO: 14 - DNA, 20 bp, synthetic construct
  misc_feature 1..20: note = Description of the artificial sequence: base sequence of primer for amplification of lacY downstream 1
  source 1..20: mol_type = other DNA
gtttccgctctgtttgctgc

SEQ ID NO: 15 - DNA, 42 bp, synthetic construct
  misc_feature 1..42: note = Description of the artificial sequence: base sequence of primer for amplification of lacZ upstream 2
  source 1..42: mol_type = other DNA
ccgttatgatatgttggtcgagctgtttcctgtgtgaaattg

SEQ ID NO: 16 - DNA, 22 bp, synthetic construct
  misc_feature 1..22: note = Description of the artificial sequence: base sequence of primer for amplification of lacY downstream 2
  source 1..22: mol_type = other DNA
cgaccaacatatcataacggag

SEQ ID NO: 17 - DNA, 41 bp, synthetic construct
  misc_feature 1..41: note = Description of the artificial sequence: base sequence of primer for amplification of yhbJ upstream 1
  source 1..41: mol_type = other DNA
ggtgcccttaaacgcctggtgtactgtttctcctcacaacg

SEQ ID NO: 18 - DNA, 23 bp, synthetic construct
  misc_feature 1..23: note = Description of the artificial sequence: base sequence of primer for amplification of yhbJ upstream 1
  source 1..23: mol_type = other DNA
agtaccgagagtctttatccatt

SEQ ID NO: 19 - DNA, 43 bp, synthetic construct
  misc_feature 1..43: note = Description of the artificial sequence: base sequence of primer for amplification of yhbJ downstream 1
  source 1..43: mol_type = other DNA
gcaggcaaatggctaaccgtaatgaccgtcaagcaaactgttg

SEQ ID NO: 20 - DNA, 21 bp, synthetic construct
  misc_feature 1..21: note = Description of the artificial sequence: base sequence of primer for amplification of yhbJ downstream 1
  source 1..21: mol_type = other DNA
gcagacaacaccacttcgacc

SEQ ID NO: 21 - DNA, 41 bp, synthetic construct
  misc_feature 1..41: note = Description of the artificial sequence: base sequence of primer for amplification of yhbJ upstream 2
  source 1..41: mol_type = other DNA
acagtttgcttgacggtcatgtactgtttctcctcacaacg

SEQ ID NO: 22 - DNA, 22 bp, synthetic construct
  misc_feature 1..22: note = Description of the artificial sequence: base sequence of primer for amplification of yhbJ downstream 2
  source 1..22: mol_type = other DNA
atgaccgtcaagcaaactgttg

SEQ ID NO: 23 - DNA, 34 bp, synthetic construct
  misc_feature 1..34: note = Description of the artificial sequence: base sequence of primer for amplification of NplgtA fragment
  source 1..34: mol_type = other DNA
gaggagaaattaaccatgcagccgctggtgagcg

SEQ ID NO: 24 - DNA, 43 bp, synthetic construct
  misc_feature 1..43: note = Description of the artificial sequence: base sequence of primer for amplification of NplgtA fragment
  source 1..43: mol_type = other DNA
aatggatttccttacgcgaattagatttcttgctctttacccg

SEQ ID NO: 25 - DNA, 23 bp, synthetic construct
  misc_feature 1..23: note = Description of the artificial sequence: base sequence of primer for amplification of lacY fragment
  source 1..23: mol_type = other DNA
ttcgcgtaaggaaatccattatg

SEQ ID NO: 26 - DNA, 38 bp, synthetic construct
  misc_feature 1..38: note = Description of the artificial sequence: base sequence of primer for amplification of lacY fragment
  source 1..38: mol_type = other DNA
atggtgatggtgatgttaagcgacttcattcacctgac

SEQ ID NO: 27 - DNA, 24 bp, synthetic construct
  misc_feature 1..24: note = Description of the artificial sequence: base sequence of primer for amplification of pUAKQE31
  source 1..24: mol_type = other DNA
ggttaatttctcctctttaatatc

SEQ ID NO: 28 - DNA, 22 bp, synthetic construct
  misc_feature 1..22: note = Description of the artificial sequence: base sequence of primer for amplification of pUAKQE31
  source 1..22: mol_type = other DNA
catcaccatcaccatcactaag

SEQ ID NO: 29 - DNA, 22 bp, synthetic construct
  misc_feature 1..22: note = Description of the artificial sequence: base sequence of primer for amplification of pSTV29
  source 1..22: mol_type = other DNA
agctgtttcctgtgtgaaattg

SEQ ID NO: 30 - DNA, 20 bp, synthetic construct
  misc_feature 1..20: note = Description of the artificial sequence: base sequence of primer for amplification of pSTV29
  source 1..20: mol_type = other DNA
gaattcactggccgtcgttt

SEQ ID NO: 31 - DNA, 38 bp, synthetic construct
  misc_feature 1..38: note = Description of the artificial sequence: base sequence of primer for amplification of ydeA fragment
  source 1..38: mol_type = other DNA
acacaggaaacagctatgacaacaaacactgtttcccg

SEQ ID NO: 32 - DNA, 36 bp, synthetic construct
  misc_feature 1..36: note = Description of the artificial sequence: base sequence of primer for amplification of ydeA fragment
  source 1..36: mol_type = other DNA
acggccagtgaattcctattgcgtctgttcttcgag

SEQ ID NO: 33 - DNA, 38 bp, synthetic construct
  misc_feature 1..38: note = Description of the artificial sequence: base sequence of primer for amplification of mdfA fragment
  source 1..38: mol_type = other DNA
acacaggaaacagctatgcaaaataaattagcttccgg

SEQ ID NO: 34 - DNA, 36 bp, synthetic construct
  misc_feature 1..36: note = Description of the artificial sequence: base sequence of primer for amplification of mdfA fragment
  source 1..36: mol_type = other DNA
acggccagtgaattcttacccttcgtgagaatttcc

SEQ ID NO: 35 - DNA, 37 bp, synthetic construct
  misc_feature 1..37: note = Description of the artificial sequence: base sequence of primer for amplification of setC fragment
  source 1..37: mol_type = other DNA
acacaggaaacagctatgcaaaaaacggctaccactc

SEQ ID NO: 36 - DNA, 39 bp, synthetic construct
  misc_feature 1..39: note = Description of the artificial sequence: base sequence of primer for amplification of setC fragment
  source 1..39: mol_type = other DNA
acggccagtgaattcctaaatatctttaataaacagcag

SEQ ID NO: 37 - DNA, 37 bp, synthetic construct
  misc_feature 1..37: note = Description of the artificial sequence: base sequence of primer for amplification of ynfM fragment
  source 1..37: mol_type = other DNA
acacaggaaacagctatgagccgtactacaactgttg

SEQ ID NO: 38 - DNA, 34 bp, synthetic construct
  misc_feature 1..34: note = Description of the artificial sequence: base sequence of primer for amplification of ynfM fragment
  source 1..34: mol_type = other DNA
acggccagtgaattctcaggcgtgcagacgacga

SEQ ID NO: 39 - DNA, 35 bp, synthetic construct
  misc_feature 1..35: note = Description of the artificial sequence: base sequence of primer for amplification of mdtD fragment
  source 1..35: mol_type = other DNA
acacaggaaacagctatgacagatcttcccgacag

SEQ ID NO: 40 - DNA, 35 bp, synthetic construct
  misc_feature 1..35: note = Description of the artificial sequence: base sequence of primer for amplification of mdtD fragment
  source 1..35: mol_type = other DNA
acggccagtgaattctcattgcgcgctcctttttc

SEQ ID NO: 41 - DNA, 36 bp, synthetic construct
  misc_feature 1..36: note = Description of the artificial sequence: base sequence of primer for amplification of yfcJ fragment
  source 1..36: mol_type = other DNA
acacaggaaacagctatgactgctgtaagccaaacc

SEQ ID NO: 42 - DNA, 36 bp, synthetic construct
  misc_feature 1..36: note = Description of the artificial sequence: base sequence of primer for amplification of yfcJ fragment
  source 1..36: mol_type = other DNA
acggccagtgaattcttaaccccgacgaaatgacag

SEQ ID NO: 43 - DNA, 38 bp, synthetic construct
  misc_feature 1..38: note = Description of the artificial sequence: base sequence of primer for amplification of emrD fragment
  source 1..38: mol_type = other DNA
acacaggaaacagctatgaaaaggcaaagaaacgtcaa

SEQ ID NO: 44 - DNA, 35 bp, synthetic construct
  misc_feature 1..35: note = Description of the artificial sequence: base sequence of primer for amplification of emrD fragment
  source 1..35: mol_type = other DNA
acggccagtgaattcttaaacgggctgcccctgat

SEQ ID NO: 45 - DNA, 39 bp, synthetic construct
  misc_feature 1..39: note = Description of the artificial sequence: base sequence of primer for amplification of ydhC fragment
  source 1..39: mol_type = other DNA
acacaggaaacagctatgcaacctgggaaaagattttta

SEQ ID NO: 46 - DNA, 36 bp, synthetic construct
  misc_feature 1..36: note = Description of the artificial sequence: base sequence of primer for amplification of ydhC fragment
  source 1..36: mol_type = other DNA
acggccagtgaattctcagtgtgattcgctatgagc

SEQ ID NO: 47 - DNA, 37 bp, synthetic construct
  misc_feature 1..37: note = Description of the artificial sequence: base sequence of primer for amplification of ybdA fragment
  source 1..37: mol_type = other DNA
acacaggaaacagctatgaataaacaatcctggctgc

SEQ ID NO: 48 - DNA, 36 bp, synthetic construct
  misc_feature 1..36: note = Description of the artificial sequence: base sequence of primer for amplification of ybdA fragment
  source 1..36: mol_type = other DNA
acggccagtgaattcttaactgtcggacgctgtcac

SEQ ID NO: 49 - DNA, 36 bp, synthetic construct
  misc_feature 1..36: note = Description of the artificial sequence: base sequence of primer for amplification of ydeE fragment
  source 1..36: mol_type = other DNA
acacaggaaacagctatgaacttatccctacgacgc

SEQ ID NO: 50 - DNA, 34 bp, synthetic construct
  misc_feature 1..34: note = Description of the artificial sequence: base sequence of primer for amplification of ydeE fragment
  source 1..34: mol_type = other DNA
acggccagtgaattctcaacaaagcgcgggctgc

SEQ ID NO: 51 - DNA, 35 bp, synthetic construct
  misc_feature 1..35: note = Description of the artificial sequence: base sequence of primer for amplification of mhpT fragment
  source 1..35: mol_type = other DNA
acacaggaaacagctatgtcgactcgtaccccttc

SEQ ID NO: 52 - DNA, 33 bp, synthetic construct
  misc_feature 1..33: note = Description of the artificial sequence: base sequence of primer for amplification of mhpT fragment
  source 1..33: mol_type = other DNA
acggccagtgaattctcaggcatcggcgcacgg

SEQ ID NO: 53 - DNA, 37 bp, synthetic construct
  misc_feature 1..37: note = Description of the artificial sequence: base sequence of primer for amplification of kgtP fragment
  source 1..37: mol_type = other DNA
acacaggaaacagctatggctgaaagtactgtaacgg

SEQ ID NO: 54 - DNA, 35 bp, synthetic construct
  misc_feature 1..35: note = Description of the artificial sequence: base sequence of primer for amplification of kgtP fragment
  source 1..35: mol_type = other DNA
acggccagtgaattcctaaagacgcatccccttcc

SEQ ID NO: 55 - DNA, 45 bp, synthetic construct
  misc_feature 1..45: note = Description of the artificial sequence: base sequence of primer for amplification of ydeA upstream 1
  source 1..45: mol_type = other DNA
ggtgcccttaaacgcctggtgttgcgaaaaagtgatgaaatgatc

SEQ ID NO: 56 - DNA, 24 bp, synthetic construct
  misc_feature 1..24: note = Description of the artificial sequence: base sequence of primer for amplification of ydeA upstream 1
  source 1..24: mol_type = other DNA
aggttcagtttaaactcacttatc

SEQ ID NO: 57 - DNA, 41 bp, synthetic construct
  misc_feature 1..41: note = Description of the artificial sequence: base sequence of primer for amplification of ydeA downstream 1
  source 1..41: mol_type = other DNA
gcaggcaaatggctaaccgtattgaaaggcccattcgggcc

SEQ ID NO: 58 - DNA, 22 bp, synthetic construct
  misc_feature 1..22: note = Description of the artificial sequence: base sequence of primer for amplification of ydeA downstream 1
  source 1..22: mol_type = other DNA
agatactcgttaagcaggcgat

SEQ ID NO: 59 - DNA, 42 bp, synthetic construct
  misc_feature 1..42: note = Description of the artificial sequence: base sequence of primer for amplification of ydeA upstream 2
  source 1..42: mol_type = other DNA
tcattaaaacgtaccattaaaacagattatcgggtgagttgc

SEQ ID NO: 60 - DNA, 25 bp, synthetic construct
  misc_feature 1..25: note = Description of the artificial sequence: base sequence of primer for amplification of ydeA downstream 2
  source 1..25: mol_type = other DNA
ttaatggtacgttttaatgatttcc

SEQ ID NO: 61 - DNA, 38 bp, synthetic construct
  misc_feature 1..38: note = Description of the artificial sequence: base sequence of primer for amplification of Cvbeta3galT fragment
  source 1..38: mol_type = other DNA
gaggagaaattaaccatggacaccatcatgattaaacg

SEQ ID NO: 62 - DNA, 60 bp, synthetic construct
  misc_feature 1..60: note = Description of the artificial sequence: base sequence of primer for amplification of Cvbeta3galT fragment
  source 1..60: mol_type = other DNA
caccagcggctgcatggttaatttctcctctttaattcattttttgatgaagcgcacata

SEQ ID NO: 63 - DNA, 19 bp, synthetic construct
  misc_feature 1..19: note = Description of the artificial sequence: base sequence of primer for amplification of pLNTII fragment
  source 1..19: mol_type = other DNA
atgcagccgctggtgagcg

SEQ ID NO: 64 - DNA, 1179 bp, Escherichia coli
  source 1..1179: mol_type = genomic DNA
atgatctggataatgacgatggctcgccgtatgaacggtgtttacgcggcatttatgctggtcgcttttatgatgggggtggccggggcgctacaggctcctacattgagcttatttctgagtcgtgaggttggcgcgcaacctttctggatcggcctcttttatacggtgaatgctattgctgggatcggcgtaagcctctggttggcaaaacgttctgacagtcagggcgatcggcgaaaactgattatattttgctgtttgatggctatcggcaatgcgctattgtttgcatttaatcgtcattatctgacgcttatcacctgtggtgtgcttctggcatctctggccaatacggcaatgccacagttatttgctctggcgcgggaatatgcggataactcggcgcgagaagtggtgatgtttagctcggtgatgcgtgcgcagctttctctggcatgggttatcggtccaccgttggcctttatgctggcgttgaattacggctttacggtgatgttttcgattgccgccgggatattcacactcagtctggtattgattgcatttatgcttccgtctgtggcgcgggtagaactgccgtcggaaaatgctttatcaatgcaaggtggctggcaggatagtaacgtacggatgttatttgtcgcctcgacgttaatgtggacctgcaacaccatgtacattattgatatgccgttgtggatcagtagcgagttaggattgccagacaaactggcgggtttcctgatggggacggcagctggactggaaataccagcaatgattctggctggctactatgtcaaacgttatggtaagcggcgaatgatggtcatagcagtggcggcaggagtactgttttacaccggattgattttctttaatagccgtatggcgttgatgacgctgcaactttttaacgctgtatttatcggcattgttgcgggtattgggatgctatggtttcaggatttaatgcctggaagagcgggggcagctaccaccttatttactaacagtatttctaccggggtaattctggctggcgttattcagggagcaattgcacaaagttgggggcactttgctgtctactgggtaattgcggttatttctgttgtcgcattatttttaaccgcaaaggttaaagacgtttga

SEQ ID NO: 65 - protein, 392 aa, Escherichia coli
MIWIMTMARRMNGVYAAFMLVAFMMGVAGALQAPTLSLFLSREVGAQPFWIGLFYTVNAIAGIGVSLWLAKRSDSQGDRRKLIIFCCLMAIGNALLFAFNRHYLTLITCGVLLASLANTAMPQLFALAREYADNSAREVVMFSSVMRAQLSLAWVIGPPLAFMLALNYGFTVMFSIAAGIFTLSLVLIAFMLPSVARVELPSENALSMQGGWQDSNVRMLFVASTLMWTCNTMYIIDMPLWISSELGLPDKLAGFLMGTAAGLEIPAMILAGYYVKRYGKRRMMVIAVAAGVLFYTGLIFFNSRMALMTLQLFNAVFIGIVAGIGMLWFQDLMPGRAGAATTLFTNSISTGVILAGVIQGAIAQSWGHFAVYWVIAVISVVALFLTAKVKDV

SEQ ID NO: 66 - DNA, 1182 bp, Escherichia coli
  source 1..1182: mol_type = genomic DNA
atgcataactcccccgcagtctccagcgcgaaatcgtttgacctgacctcgacggcgtttttaatcgttgcctttctcaccggtattgcgggcgctctgcaaaccccgacactcagtatttttcttaccgatgaagtacatgcccgtccggcgatggtgggattcttctttaccggcagcgctgtcattgggattctggtaagtcagtttctcgccgggcgctctgataagcgcggcgatcgcaaatcgctgattgtcttttgctgcctgttaggcgtgctggcctgcaccctttttgcctggaatcgcaactactttgttttgctattcgttggcgtctttcttagcagctttggctcgaccgctaacccgcaaatgtttgcccttgcccgtgaacatgccgacaaaaccggacgtgaggcggtgatgttcagctcttttttacgcgctcaggtttcactggcatgggtcattggcccaccgctggcttatgccttagcgatgggtttcagctttacggtaatgtatctgagcgcagcggtagcgtttattgtttgcggtgtgatggtgtggctgtttttaccgtcgatgcgaaaagagcttccgctggcgaccggcacgatcgaagcgccgcgccgtaaccgtcgcgatacgctgctgctgtttgtcatttgtacattgatgtggggctcgaacagcctgtacatcatcaacatgccgctatttattatcaacgaactgcatcttcccgagaaactggccggtgtgatgatggggaccgccgccgggctggaaatcccgacgatgttgattgccggatatttcgccaaacgtctgggtaagcgtttcttaatgcgcgttgctgccgtgggtggcgtctgtttttacgcaggaatgctgatggcgcattcacctgtcattctgttgggcttgcagctgctaaatgctatttttattggcattctgggcggcatcgggatgctctattttcaggatctgatgcccggtcaggcgggttcagccaccacgctctataccaacacttcgcgcgtgggctggatcatcgcaggatcagtggcgggcatcgtcgccgagatctggaattatcacgctgtgttctggtttgcgatggtgatgattatcgccactctgttttgcttactgcggattaaagatgtttaa

SEQ ID NO: 67 - protein, 393 aa, Escherichia coli
MHNSPAVSSAKSFDLTSTAFLIVAFLTGIAGALQTPTLSIFLTDEVHARPAMVGFFFTGSAVIGILVSQFLAGRSDKRGDRKSLIVFCCLLGVLACTLFAWNRNYFVLLFVGVFLSSFGSTANPQMFALAREHADKTGREAVMFSSFLRAQVSLAWVIGPPLAYALAMGFSFTVMYLSAAVAFIVCGVMVWLFLPSMRKELPLATGTIEAPRRNRRDTLLLFVICTLMWGSNSLYIINMPLFIINELHLPEKLAGVMMGTAAGLEIPTMLIAGYFAKRLGKRFLMRVAAVGGVCFYAGMLMAHSPVILLGLQLLNAIFIGILGGIGMLYFQDLMPGQAGSATTLYTNTSRVGWIIAGSVAGIVAEIWNYHAVFWFAMVMIIATLFCLLRIKDV